European Patent Application EP 4 410 838 A1, published August 7, 2024. Title: 抗CD39抗体-药物偶联物及其用途. Applicant: 杭州邦顺制药有限公司. The sequence listing filed with the application follows.

SEQUENCE LISTING (19 sequences)

SEQ ID NO: 1 - protein, 5 aa, synthetic construct
NYWMY

SEQ ID NO: 2 - protein, 17 aa, synthetic construct
RIAPSSGATKYNEKFKN

SEQ ID NO: 3 - protein, 13 aa, synthetic construct
SGIYYDYDWFFDV

SEQ ID NO: 4 - protein, 11 aa, synthetic construct
KASQDINKYIG

SEQ ID NO: 5 - protein, 7 aa, synthetic construct
YTSTLQP

SEQ ID NO: 6 - protein, 9 aa, synthetic construct
LQYHALLFT

SEQ ID NO: 7 - protein, 122 aa, synthetic construct
QVQLQQPGAELVKPGASVKLSCKTSGYTFTNYWMYWVKHRPGRGLEWIGRIAPSSGATKYNEKFKNKATLTVDKPSSTAYMQLSSLTSEDSAVYYCARSGIYYDYDWFFDVSGTGTTVTVSS

SEQ ID NO: 8 - protein, 107 aa, synthetic construct
DIQMTQSPSSLSASLGGKVTITCKASQDINKYIGWYQHAPGKGPRLLIHYTSTLQPGIPSRFSGSGSGRDYSLSISNLEPEDIATYYCLQYHALLFTFGSGTKLELK

SEQ ID NO: 9 - protein, 449 aa, synthetic construct
QVQLQQPGAELVKPGASVKLSCKTSGYTFTNYWMYWVKHRPGRGLEWIGRIAPSSGATKYNEKFKNKATLTVDKPSSTAYMQLSSLTSEDSAVYYCARSGIYYDYDWFFDVSGTGTTVTVSSASTKGPSVFPLAPCSRSTSESTAALGCLVKDYFPEPVTVSWNSGALTSGVHTFPAVLQSSGLYSLSSVVTVPSSSLGTKTYTCNVDHKPSNTKVDKRVESKYGPPCPPCPAPEFLGGPSVFLFPPKPKDTLMISRTPEVTCVVVDVSQEDPEVQFNWYVDGVEVHNAKTKPREEQFNSTYRVVSVLTVLHQDWLNGKEYKCKVSNKGLPSSIEKTISKAKGQPREPQVYTLPPSQEEMTKNQVSLTCLVKGFYPSDIAVEWESNGQPENNYKTTPPVLDSDGSFFLYSRLTVDKSRWQEGNVFSCSVMHEALHNHYTQKSLSLSLGK

SEQ ID NO: 10 - protein, 214 aa, synthetic construct
DIQMTQSPSSLSASLGGKVTITCKASQDINKYIGWYQHAPGKGPRLLIHYTSTLQPGIPSRFSGSGSGRDYSLSISNLEPEDIATYYCLQYHALLFTFGSGTKLELKRTVAAPSVFIFPPSDEQLKSGTASVVCLLNNFYPREAKVQWKVDNALQSGNSQESVTEQDSKDSTYSLSSTLTLSKADYEKHKVYACEVTHQGLSSPVTKSFNRGEC

SEQ ID NO: 11 - protein, 122 aa, synthetic construct
QVQLVQSGAEVKKPGASVKVSCKASGYTFTNYWMYWVRQAPGQGLEWMGRIAPSSGATKYNEKFKNRVTMTRDTSISTAYMELSRLRSDDTAVYYCARSGIYYDYDWFFDVWGQGTTVTVSS

SEQ ID NO: 12 - protein, 122 aa, synthetic construct
QVQLVQSGAEVKKPGASVKVSCKASGYTFTNYWMYWVRQAPGQGLEWMGRIAPSSGATKYNEKFKNRVTLTVDTSISTAYMELSRLRSDDTAVYYCARSGIYYDYDWFFDVWGQGTTVTVSS

SEQ ID NO: 13 - protein, 122 aa, synthetic construct
QVQLVQSGAEVKKPGASVKVSCKASGYTFTNYWMYWVRQAPGQGLEWIGRIAPSSGATKYNEKFKNRATLTVDTSISTAYMELSRLRSDDTAVYYCARSGIYYDYDWFFDVWGQGTTVTVSS

SEQ ID NO: 14 - protein, 122 aa, synthetic construct
QVQLVQSGAEVKKPGASVKVSCKASGYTFTNYWMYWVRQRPGRGLEWIGRIAPSSGATKYNEKFKNRATLTVDTSISTAYMELSRLRSDDTAVYYCARSGIYYDYDWFFDVWGQGTTVTVSS

SEQ ID NO: 15 - protein, 122 aa, synthetic construct
QVQLVQSGAEVKKPGASVKVSCKASGYTFTNYWMYWVRQRPGRGLEWIGRIAPSSGATKYNEKFKNRATLTVDTSISTAYMELSRLRSDDTAVYYCARSGIYYDYDWFFDVSGQGTTVTVSS

SEQ ID NO: 16 - protein, 107 aa, synthetic construct
DIQMTQSPSSLSASVGDRVTITCKASQDINKYIGWYQQKPGKAPKLLIHYTSTLQPGVPSRFSGSGSGTDFTFTISSLQPEDIATYYCLQYHALLFTFGQGTKLEIK

SEQ ID NO: 17 - protein, 107 aa, synthetic construct
DIQMTQSPSSLSASVGDRVTITCKASQDINKYIGWYQQKPGKAPKLLIHYTSTLQPGVPSRFSGSGSGRDYTFTISSLQPEDIATYYCLQYHALLFTFGQGTKLEIK

SEQ ID NO: 18 - protein, 327 aa, synthetic construct
ASTKGPSVFPLAPCSRSTSESTAALGCLVKDYFPEPVTVSWNSGALTSGVHTFPAVLQSSGLYSLSSVVTVPSSSLGTKTYTCNVDHKPSNTKVDKRVESKYGPPCPPCPAPEFLGGPSVFLFPPKPKDTLMISRTPEVTCVVVDVSQEDPEVQFNWYVDGVEVHNAKTKPREEQFNSTYRVVSVLTVLHQDWLNGKEYKCKVSNKGLPSSIEKTISKAKGQPREPQVYTLPPSQEEMTKNQVSLTCLVKGFYPSDIAVEWESNGQPENNYKTTPPVLDSDGSFFLYSRLTVDKSRWQEGNVFSCSVMHEALHNHYTQKSLSLSLGK

SEQ ID NO: 19 - protein, 107 aa, synthetic construct [sequence omitted]